European Patent Application EP 4 725 963 A1, published April 15, 2026. Title: 抗NPR1抗体及其医药用途. Applicant: 江苏恒瑞医药股份有限公司. Application WO. The sequence listing filed with the application follows.

SEQUENCE LISTING (128 sequences)

SEQ ID NO: 1 - protein, 673 aa, synthetic construct
  CHAIN 1..673: note = hNPR1-hFc
GNLTVAVVLPLANTSYPWSWARVGPAVELALAQVKARPDLLPGWTVRTVLGSSENALGVCSDTAAPLAAVDLKWEHNPAVFLGPGCVYAAAPVGRFTAHWRVPLLTAGAPALGFGVKDEYALTTRAGPSYAKLGDFVAALHRRLGWERQALMLYAYRPGDEEHCFFLVEGLFMRVRDRLNITVDHLEFAEDDLSHYTRLLRTMPRKGRVIYICSSPDAFRTLMLLALEAGLCGEDYVFFHLDIFGQSLQGGQGPAPRRPWERGDGQDVSARQAFQAAKIITYKDPDNPEYLEFLKQLKHLAYEQFNFTMEDGLVNTIPASFHDGLLLYIQAVTETLAHGGTVTDGENITQRMWNRSFQGVTGYLKIDSSGDRETDFSLWDMDPENGAFRVVLNYNGTSQELVAVSGRKLNWPLGYPPPDIPKCGFDNEDPACNQDHLSTLEEPKSSDKTHTCPPCPAPELLGGPSVFLFPPKPKDTLMISRTPEVTCVVVDVSHEDPEVKFNWYVDGVEVHNAKTKPREEQYNSTYRVVSVLTVLHQDWLNGKEYKCKVSNKALPAPIEKTISKAKGQPREPQVYTLPPSRDELTKNQVSLTCLVKGFYPSDIAVEWESNGQPENNYKTTPPVLDSDGSFFLYSKLTVDKSRWQQGNVFSCSVMHEALHNHYTQKSLSLSPGK

SEQ ID NO: 2 - protein, 673 aa, synthetic construct
  CHAIN 1..673: note = cNPR1-hFc
GNLTVAVVLPLANTSYPWSWARVGPAVELALARVKARPDLLPGWTVRTVLGSSENALGVCSDTAAPLAAVDLKWEHNPAAFLGPGCVYAAAPVGRFTAHWRVPLLTAGAPALGFGVKDEYALTTRAGPSYAKLGDFVAALHRRLGWERQALMLYAYRPGDEEHCFFLVEGLFMRVRDRLNITVDHLEFAEDDLSHYTRLLRTMPRKGRVIYICSSPDAFRTLMLLALEAGLCGEDYVFFHLDIFGQSLQGGQGPAPRRPWERGDGQDVSARQAFQAAKIITYKEPDNPEYLEFLKQLKHLAREQFNFTMEDGLVNTIPASFHDGLLLYIQAVTETLAHGGTVTDGENITQRMWNRSFQGVTGYLKIDSSGDRETDFSLWDMDPETGAFRVVLNYNGTSQELVAVSGRKLNWPLGYPPPDIPKCGFDNEDPACNQDHLSTLEEPKSSDKTHTCPPCPAPELLGGPSVFLFPPKPKDTLMISRTPEVTCVVVDVSHEDPEVKFNWYVDGVEVHNAKTKPREEQYNSTYRVVSVLTVLHQDWLNGKEYKCKVSNKALPAPIEKTISKAKGQPREPQVYTLPPSRDELTKNQVSLTCLVKGFYPSDIAVEWESNGQPENNYKTTPPVLDSDGSFFLYSKLTVDKSRWQQGNVFSCSVMHEALHNHYTQKSLSLSPGK

SEQ ID NO: 3 - protein, 673 aa, synthetic construct
  CHAIN 1..673: note = rNPR1-hFc
SDLTVAVVLPLTNTSYPWSWARVGPAVELALARVKARPDLLPGWTVRMVLGSSENAAGVCSDTAAPLAAVDLKWEHSPAVFLGPGCVYSAAPVGRFTAHWRVPLLTAGAPALGIGVKDEYALTTRTGPSHVKLGDFVTALHRRLGWEHQALVLYADRLGDDRPCFFIVEGLYMRVRERLNITVNHQEFVEGDPDHYPKLLRAVRRKGRVIYICSSPDAFRNLMLLALNAGLTGEDYVFFHLDVFGQSLKSAQGLVPQKPWERGDGQDRSARQAFQAAKIITYKEPDNPEYLEFLKQLKLLADKKFNFTVEDGLKNIIPASFHDGLLLYVQAVTETLAQGGTVTDGENITQRMWNRSFQGVTGYLKIDRNGDRDTDFSLWDMDPETGAFRVVLNYNGTSQELMAVSEHKLYWPLGYPPPDVPKCGFDNEDPACNQDHFSTLEEPKSSDKTHTCPPCPAPELLGGPSVFLFPPKPKDTLMISRTPEVTCVVVDVSHEDPEVKFNWYVDGVEVHNAKTKPREEQYNSTYRVVSVLTVLHQDWLNGKEYKCKVSNKALPAPIEKTISKAKGQPREPQVYTLPPSRDELTKNQVSLTCLVKGFYPSDIAVEWESNGQPENNYKTTPPVLDSDGSFFLYSKLTVDKSRWQQGNVFSCSVMHEALHNHYTQKSLSLSPGK

SEQ ID NO: 4 - protein, 1061 aa, Homo sapiens
  CHAIN 1..1061: note = hNPR1
MPGPRRPAGSRLRLLLLLLLPPLLLLLRGSHAGNLTVAVVLPLANTSYPWSWARVGPAVELALAQVKARPDLLPGWTVRTVLGSSENALGVCSDTAAPLAAVDLKWEHNPAVFLGPGCVYAAAPVGRFTAHWRVPLLTAGAPALGFGVKDEYALTTRAGPSYAKLGDFVAALHRRLGWERQALMLYAYRPGDEEHCFFLVEGLFMRVRDRLNITVDHLEFAEDDLSHYTRLLRTMPRKGRVIYICSSPDAFRTLMLLALEAGLCGEDYVFFHLDIFGQSLQGGQGPAPRRPWERGDGQDVSARQAFQAAKIITYKDPDNPEYLEFLKQLKHLAYEQFNFTMEDGLVNTIPASFHDGLLLYIQAVTETLAHGGTVTDGENITQRMWNRSFQGVTGYLKIDSSGDRETDFSLWDMDPENGAFRVVLNYNGTSQELVAVSGRKLNWPLGYPPPDIPKCGFDNEDPACNQDHLSTLEVLALVGSLSLLGILIVSFFIYRKMQLEKELASELWRVRWEDVEPSSLERHLRSAGSRLTLSGRGSNYGSLLTTEGQFQVFAKTAYYKGNLVAVKRVNRKRIELTRKVLFELKHMRDVQNEHLTRFVGACTDPPNICILTEYCPRGSLQDILENESITLDWMFRYSLTNDIVKGMLFLHNGAICSHGNLKSSNCVVDGRFVLKITDYGLESFRDLDPEQGHTVYAKKLWTAPELLRMASPPVRGSQAGDVYSFGIILQEIALRSGVFHVEGLDLSPKEIIERVTRGEQPPFRPSLALQSHLEELGLLMQRCWAEDPQERPPFQQIRLTLRKFNRENSSNILDNLLSRMEQYANNLEELVEERTQAYLEEKRKAEALLYQILPHSVAEQLKRGETVQAEAFDSVTIYFSDIVGFTALSAESTPMQVVTLLNDLYTCFDAVIDNFDVYKVETIGDAYMVVSGLPVRNGRLHACEVARMALALLDAVRSFRIRHRPQEQLRLRIGIHTGPVCAGVVGLKMPRYCLFGDTVNTASRMESNGEALKIHLSSETKAVLEEFGGFELELRGDVEMKGKGKVRTYWLLGERGSSTRG

SEQ ID NO: 5 - protein, 1061 aa, Macaca fascicularis
  CHAIN 1..1061: note = cNPR1
MPGPRRPAGSRLRLLLLLLLPPLLLLLRGSHAGNLTVAVVLPLANTSYPWSWARVGPAVELALARVKARPDLLPGWTVRTVLGSSENALGVCSDTAAPLAAVDLKWEHNPAAFLGPGCVYAAAPVGRFTAHWRVPLLTAGAPALGFGVKDEYALTTRAGPSYAKLGDFVAALHRRLGWERQALMLYAYRPGDEEHCFFLVEGLFMRVRDRLNITVDHLEFAEDDLSHYTRLLRTMPRKGRVIYICSSPDAFRTLMLLALEAGLCGEDYVFFHLDIFGQSLQGGQGPAPRRPWERGDGQDVSARQAFQAAKIITYKEPDNPEYLEFLKQLKHLAREQFNFTMEDGLVNTIPASFHDGLLLYIQAVTETLAHGGTVTDGENITQRMWNRSFQGVTGYLKIDSSGDRETDFSLWDMDPETGAFRVVLNYNGTSQELVAVSGRKLNWPLGYPPPDIPKCGFDNEDPACNQDHLSTLEVLALVGSLSLLSILIVSFFIYRKMQLEKELASELWRVRWEDVEPSSLERHLRSAGSRLTLSGRGSNYGSLLTTEGQFQVFAKTAYYKGNLVAVKRVNRKRIELTRKVLFELKHMRDVQNEHLTRFVGACTDPPNICILTEYCPRGSLQDILENESITLDWMFRYSLTNDIVKGMLFLHNGAICSHGNLKSSNCVVDGRFVLKITDYGLESFRDLDPEQGHTLYAKKLWTAPELLRMASPPVRGSQAGDIYSFGIILQEIALRSGVFHVEGLDLSPKEIIERVTRGEQPPFRPSLALQSHLEELGLLMQRCWAEDPQERPPFQQIRLTLRKFNRENSSNILDNLLSRMEQYANNLEELVEERTQAYLEEKRKAEALLYQILPHSVAEQLKRGETVQAEAFDSVTIYFSDIVGFTALSAESTPMQVVTLLNDLYTCFDAVIDNFDVYKVETIGDAYMVVSGLPVRNGRLHACEVARMALALLDAVRSFRIRHRPQEQLRLRIGIHTGPVCAGVVGLKMPRYCLFGDTVNTASRMESNGEALKIHLSSETKAVLEEFGGFELELRGDVEMKGKGKVRTYWLLGERGSSTRG

SEQ ID NO: 6 - protein, 1057 aa, Rattus norvegicus
  CHAIN 1..1057: note = rNPR1
MPGSRRVRPRLRALLLLPPLLLLRGGHASDLTVAVVLPLTNTSYPWSWARVGPAVELALARVKARPDLLPGWTVRMVLGSSENAAGVCSDTAAPLAAVDLKWEHSPAVFLGPGCVYSAAPVGRFTAHWRVPLLTAGAPALGIGVKDEYALTTRTGPSHVKLGDFVTALHRRLGWEHQALVLYADRLGDDRPCFFIVEGLYMRVRERLNITVNHQEFVEGDPDHYPKLLRAVRRKGRVIYICSSPDAFRNLMLLALNAGLTGEDYVFFHLDVFGQSLKSAQGLVPQKPWERGDGQDRSARQAFQAAKIITYKEPDNPEYLEFLKQLKLLADKKFNFTVEDGLKNIIPASFHDGLLLYVQAVTETLAQGGTVTDGENITQRMWNRSFQGVTGYLKIDRNGDRDTDFSLWDMDPETGAFRVVLNYNGTSQELMAVSEHKLYWPLGYPPPDVPKCGFDNEDPACNQDHFSTLEVLALVGSLSLISFLIVSFFIYRKMQLEKELVSELWRVRWEDLQPSSLERHLRSAGSRLTLSGRGSNYGSLLTTEGQFQVFAKTAYYKGNLVAVKRVNRKRIELTRKVLFELKHMRDVQNEHLTRFVGACTDPPNICILTEYCPRGSLQDILENESITLDWMFRYSLTNDIVKGMLFLHNGAICSHGNLKSSNCVVDGRFVLKITDYGLESFRDPEPEQGHTLFAKKLWTAPELLRMASPPARGSQAGDVYSFGIILQEIALRSGVFYVEGLDLSPKEIIERVTRGEQPPFRPSMDLQSHLEELGQLMQRCWAEDPQERPPFQQIRLALRKFNKENSSNILDNLLSRMEQYANNLEELVEERTQAYLEEKRKAEALLYQILPHSVAEQLKRGETVQAEAFDSVTIYFSDIVGFTALSAESTPMQVVTLLNDLYTCFDAVIDNFDVYKVETIGDAYMVVSGLPVRNGQLHAREVARMALALLDAVRSFRIRHRPQEQLRLRIGIHTGPVCAGVVGLKMPRYCLFGDTVNTASRMESNGEALKIHLSSETKAVLEEFDGFELELRGDVEMKGKGKVRTYWLLGERGCSTRG

SEQ ID NO: 7 - protein, 122 aa, synthetic construct
  DOMAIN 1..122: note = NPR1-CHAb-SFM-102-1-VH
DVKLVESGEGLVKPGGSLKLSCAASGFTFSTYAMSWVRQTPEKRLEWVAYISRGGDYIYYADTVKGRFTISRDNARNTLYLQMSSLKSEDTAMYYCTRDQTTVVVHWYFDVWGTGTTVTVSS

SEQ ID NO: 8 - protein, 104 aa, synthetic construct
  DOMAIN 1..104: note = NPR1-CHAb-SFM-102-1-VL
QIVLTQSPAIMSASPGEKVTMTCSASSSINYMHWYQQKPGTSPKRWIYDTSKLASGVPARFSGSGSGTSYSLTISSMEAGDAATYYCHQRNSYTFGGGTKLEIK

SEQ ID NO: 9 - protein, 122 aa, synthetic construct
  DOMAIN 1..122: note = NPR1-CHAb-SFM-127-1 -VH
QAYLQQSGPELVKPGASVKISCKASGYSFTGYFMNWVMQSHGKSLEWIGRINPYNGDTFYNQKFKGKATLTVDKSSSTVHMELRSLASEDSAVYYCARRGYGNRGYWYFDVWGAGTTVTVSS

SEQ ID NO: 10 - protein, 111 aa, synthetic construct
  DOMAIN 1..111: note = NPR1-CHAb-SFM-127-1-VL
NIVLTQSPASLAVSLGQRATISCRASESVDSYGNSFMHWYQQKPGQPPKVLIYLASTLESGVPARFSGSGSRTDFTLTIDPVEADDAATYYCQQNNEDPLTFGAGTKLELK

SEQ ID NO: 11 - protein, 119 aa, synthetic construct
  DOMAIN 1..119: note = NPR1-CHAb-SFM-128-VH
QVQLQQSGAELAKPGASVKLSCKASGYTFTSYWMHWVKQRPGRGLEWIGRIDPNSGVTKYNEKFKSKATLTVDKPSSPAYMQLSSLTSEDSAVYYCARSSYLGRYFDVWGTGTTVTVSS

SEQ ID NO: 12 - protein, 106 aa, synthetic construct
  DOMAIN 1..106: note = NPR1-CHAb-SFM-128-VL
QIVLTQSPAIMSASPGEKVTMTCSATSSVSYMYWYQQKPGSSPRLLIYDTYNLASRVPIRFSGSGSGTSYSLTISRMEAEDAATYYCQQWSSYPPTFGSGTKLEIK

SEQ ID NO: 13 - protein, 122 aa, synthetic construct
  DOMAIN 1..122: note = NPR1-CHAb-SFM-135-VH
DVKLVESGEGLVKPGGSLKLSCVASGFSISTYGMSWVRQTPEKRLEWVAYINSGGNYIYYADTVKGRFTISRDNARNTLYLQMSSLKSEDTAMYYCTRDRTTIVVHWYFDVWGTGTTVTVSS

SEQ ID NO: 14 - protein, 103 aa, synthetic construct
  DOMAIN 1..103: note = NPR1-CHAb-SFM-135-VL
QIVLTQSPAIMSASPGEKVTMTCSASSSLNFMHWYQQKPGTSPKRWIYDTSKLASGVPARFSGSGSGTSYSLTISSMEAEDAATYYCHQRSSTFGGGTKLELK

SEQ ID NO: 15 - protein, 119 aa, synthetic construct
  DOMAIN 1..119: note = NPR1-CHAb-SFM-140-VH
QVQLQQSGAELVKPGASVKLSCKASGYTFTSYWMHWVKQRPGRGLEWIGRIDPNSGVTKYNEKFKSKVTLTVDKPSSPAYIQLSSLTSEDSAVYYCARSGGLRRYFDVWGTGTTVTVSS

SEQ ID NO: 16 - protein, 106 aa, synthetic construct
  DOMAIN 1..106: note = NPR1-CHAb-SFM-140-VL
QIVLTQSPAIMSASPGEKVTMTCSASSSVSYMYWYQQKPGSSPRLLIFDTYNLASGVPVRFSGSGSGTSYSLTINRMEAEDAATYYCQQWSSYPPTFGAGTKLELK

SEQ ID NO: 17 - protein, 5 aa, synthetic construct
  DOMAIN 1..5: note = m102-HCDR1
TYAMS

SEQ ID NO: 18 - protein, 17 aa, synthetic construct
  DOMAIN 1..17: note = m102-HCDR2
YISRGGDYIYYADTVKG

SEQ ID NO: 19 - protein, 13 aa, synthetic construct
  DOMAIN 1..13: note = m102-HCDR3
DQTTVVVHWYFDV

SEQ ID NO: 20 - protein, 10 aa, synthetic construct
  DOMAIN 1..10: note = m102-LCDR1
SASSSINYMH

SEQ ID NO: 21 - protein, 7 aa, synthetic construct
  DOMAIN 1..7: note = m102-LCDR2
DTSKLAS

SEQ ID NO: 22 - protein, 7 aa, synthetic construct
  DOMAIN 1..7: note = m102-LCDR3
HQRNSYT

SEQ ID NO: 23 - protein, 5 aa, synthetic construct
  DOMAIN 1..5: note = m127-HCDR1
GYFMN

SEQ ID NO: 24 - protein, 17 aa, synthetic construct
  DOMAIN 1..17: note = m127-HCDR2
RINPYNGDTFYNQKFKG

SEQ ID NO: 25 - protein, 13 aa, synthetic construct
  DOMAIN 1..13: note = m127-HCDR3
RGYGNRGYWYFDV

SEQ ID NO: 26 - protein, 15 aa, synthetic construct
  DOMAIN 1..15: note = m127-LCDR1
RASESVDSYGNSFMH

SEQ ID NO: 27 - protein, 7 aa, synthetic construct
  DOMAIN 1..7: note = m127-LCDR2
LASTLES

SEQ ID NO: 28 - protein, 9 aa, synthetic construct
  DOMAIN 1..9: note = m127-LCDR3
QQNNEDPLT

SEQ ID NO: 29 - protein, 5 aa, synthetic construct
  DOMAIN 1..5: note = m128-HCDR1
SYWMH

SEQ ID NO: 30 - protein, 17 aa, synthetic construct
  DOMAIN 1..17: note = m128-HCDR2
RIDPNSGVTKYNEKFKS

SEQ ID NO: 31 - protein, 10 aa, synthetic construct
  DOMAIN 1..10: note = m128-HCDR3
SSYLGRYFDV

SEQ ID NO: 32 - protein, 10 aa, synthetic construct
  DOMAIN 1..10: note = m128-LCDR1
SATSSVSYMY

SEQ ID NO: 33 - protein, 7 aa, synthetic construct
  DOMAIN 1..7: note = m128-LCDR2
DTYNLAS

SEQ ID NO: 34 - protein, 9 aa, synthetic construct
  DOMAIN 1..9: note = m128-LCDR3
QQWSSYPPT

SEQ ID NO: 35 - protein, 5 aa, synthetic construct
  DOMAIN 1..5: note = m135-HCDR1
TYGMS

SEQ ID NO: 36 - protein, 17 aa, synthetic construct
  DOMAIN 1..17: note = m135-HCDR2
YINSGGNYIYYADTVKG

SEQ ID NO: 37 - protein, 13 aa, synthetic construct
  DOMAIN 1..13: note = m135-HCDR3
DRTTIVVHWYFDV

SEQ ID NO: 38 - protein, 10 aa, synthetic construct
  DOMAIN 1..10: note = m135-LCDR1
SASSSLNFMH

SEQ ID NO: 39 - protein, 6 aa, synthetic construct
  DOMAIN 1..6: note = m135-LCDR3
HQRSST

SEQ ID NO: 40 - protein, 17 aa, synthetic construct
  DOMAIN 1..17: note = m140-HCDR2
RIDPNSGVTKYNEKFKS

SEQ ID NO: 41 - protein, 10 aa, synthetic construct
  DOMAIN 1..10: note = m140-HCDR3
SGGLRRYFDV

SEQ ID NO: 42 - protein, 10 aa, synthetic construct
  DOMAIN 1..10: note = m140-LCDR1
SASSSVSYMY

SEQ ID NO: 43 - protein, 330 aa, Homo sapiens [sequence omitted]

SEQ ID NO: 44 - protein, 107 aa, Homo sapiens [sequence omitted]

SEQ ID NO: 45 - protein, 5 aa, synthetic construct
  DOMAIN 1..5: note = hu102VH4-HCDR1
SYAMS

SEQ ID NO: 46 - protein, 17 aa, synthetic construct
  DOMAIN 1..17: note = hu102VH4-HCDR2
YISRGGDYIYYADSVKG

SEQ ID NO: 47 - protein, 210 aa, synthetic construct
  CHAIN 1..210: note = Hu135H3L1-LC
DIQLTQSPSSLSASVGDRVTITCSASSSLNFMHWYQQKPGKSPKRWIYDTSKLASGVPSRFSGSGSGTDYTLTISSLQPEDFATYYCHQRSSTFGGGTKVEIKRTVAAPSVFIFPPSDEQLKSGTASVVCLLNNFYPREAKVQWKVDNALQSGNSQESVTEQDSKDSTYSLSSTLTLSKADYEKHKVYACEVTHQGLSSPVTKSFNRGEC

SEQ ID NO: 48 - protein, 122 aa, synthetic construct
  DOMAIN 1..122: note = hu102VH1
EVQLVESGGGLVKPGGSLRLSCAASGFTFSTYAMSWVRQAPGKRLEWVSYISRGGDYIYYADTVKGRFTISRDNAKNSLYLQMNSLRAEDTAVYYCTRDQTTVVVHWYFDVWGQGTTVTVSS

SEQ ID NO: 49 - protein, 122 aa, synthetic construct
  DOMAIN 1..122: note = hu102VH2
EVQLVESGEGLVKPGGSLRLSCAASGFTFSTYAMSWVRQAPGKRLEWVAYISRGGDYIYYADTVKGRFTISRDNAKNSLYLQMNSLRAEDTAVYYCTRDQTTVVVHWYFDVWGQGTTVTVSS

SEQ ID NO: 50 - protein, 122 aa, synthetic construct
  DOMAIN 1..122: note = hu102VH3
DVKLVESGEGLVKPGGSLRLSCAASGFTFSTYAMSWVRQAPGKRLEWVAYISRGGDYIYYADTVKGRFTISRDNAKNSLYLQMNSLRAEDTAVYYCTRDQTTVVVHWYFDVWGQGTTVTVSS

SEQ ID NO: 51 - protein, 122 aa, synthetic construct
  DOMAIN 1..122: note = hu102VH4
DVKLVESGEGLVKPGGSLRLSCAASGFTFSSYAMSWVRQAPGKRLEWVAYISRGGDYIYYADSVKGRFTISRDNAKNSLYLQMNSLRAEDSAVYYCTRDQTTVVVHWYFDVWGQGTTVTVSS

SEQ ID NO: 52 - protein, 122 aa, synthetic construct
  DOMAIN 1..122: note = hu102VH5
DVKLVESGEGLVKPGGSLRLSCAASGFTFSTYGMSWVRQAPGKRLEWVAYISRGGDYIYYADTVKGRFTISRDNAKNSLYLQMNSLRAEDTAVYYCTRDQTTVVVHWYFDVWGQGTTVTVSS

SEQ ID NO: 53 - protein, 104 aa, synthetic construct
  DOMAIN 1..104: note = hu102VL3
EIVLTQSPATLSLSPGERATLSCSASSSINYMHWYQQKPGQAPRRWIYDTSKLASGVPARFSGSGSGTDYTLTISSLEPEDFAVYYCHQRNSYTFGGGTKVEIK

SEQ ID NO: 54 - protein, 104 aa, synthetic construct
  DOMAIN 1..104: note = hu102VL4
EIVLTQSPATLSLSPGERATLSCSASSSINYMHWYQQKPGQSPKRWIYDTSKLASGVPARFSGSGSGTDYTLTISSLEPEDFAVYYCHQRNSYTFGGGTKVEIK

SEQ ID NO: 55 - protein, 104 aa, synthetic construct
  DOMAIN 1..104: note = hu102VL5
DIQMTQSPSSLSASVGDRVTITCSASSSINYMHWYQQKPGKAPKRWIYDTSKLASGVPSRFSGSGSGTDFTLTISSLQPEDFATYYCHQRNSYTFGGGTKVEIK

SEQ ID NO: 56 - protein, 104 aa, synthetic construct
  DOMAIN 1..104: note = hu102VL6
DIQLTQSPSSLSASVGDRVTITCSASSSINYMHWYQQKPGKSPKRWIYDTSKLASGVPSRFSGSGSGTDYTLTISSLQPEDFATYYCHQRNSYTFGGGTKVEIK

SEQ ID NO: 57 - protein, 17 aa, synthetic construct
  DOMAIN 1..17: note = hu127VH4/ VH7/ VH8-HCDR2
RINPYSGDTFYNQKFKG

SEQ ID NO: 58 - protein, 122 aa, synthetic construct
  DOMAIN 1..122: note = hu127VH4
EAYLVQSGAEVKKPGASVKVSCKASGYSFTGYFMNWVRQAPGKGLEWMGRINPYSGDTFYNQKFKGRVTLTVDKSTSTVYMELSSLRSEDTAVYYCARRGYGNRGYWYFDVWGQGTTVTVSS

SEQ ID NO: 59 - protein, 122 aa, synthetic construct
  DOMAIN 1..122: note = hu127VH7
QVQLVQSGAEVKKPGASVKVSCKASGYTFTGYFMNWVRQAPGQGLEWMGRINPYSGDTFYNQKFKGRVTMTVDKSTSTVYMELSSLRSEDTAVYYCARRGYGNRGYWYFDVWGQGTTVTVSS

SEQ ID NO: 60 - protein, 122 aa, synthetic construct
  DOMAIN 1..122: note = hu127VH8
EVQLVQSGAEVKKPGASVKVSCKASGYTFTGYFMNWVRQAPGQGLEWMGRINPYSGDTFYNQKFKGRVTMTVDKSTSTVYMELSSLRSEDTAVYYCARRGYGNRGYWYFDVWGQGTTVTVSS

SEQ ID NO: 61 - protein, 111 aa, synthetic construct
  DOMAIN 1..111: note = hu127VL1
DIVMTQSPDSLAVSLGERATINCRASESVDSYGNSFMHWYQQKPGQPPKVLIYLASTLESGVPDRFSGSGSRTDFTLTISSLQAEDVAVYYCQQNNEDPLTFGQGTKLEIK

SEQ ID NO: 62 - protein, 111 aa, synthetic construct
  DOMAIN 1..111: note = hu127VL3
NIVLTQSPDSLAVSLGERATINCRASESVDSYGNSFMHWYQQKPGQPPKVLIYLASTLESGVPDRFSGSGSRTDFTLTISSLQAEDVAVYYCQQNNEDPLTFGQGTKLEIK

SEQ ID NO: 63 - protein, 111 aa, synthetic construct
  DOMAIN 1..111: note = hu127VL4
NIVLTQSPDSLAVSLGERATINCRASESVDSYGNSFMHWYQQKPGQPPKVLIYLASTLESGVPARFSGSGSRTDFTLTISSLEAEDVAVYYCQQNNEDPLTFGQGTKLEIK

SEQ ID NO: 64 - protein, 111 aa, synthetic construct
  DOMAIN 1..111: note = hu127VL5
NIQLTQSPSSLSASVGDRVTITCRASESVDSYGNSFMHWYQQKPGKAPKVLIYLASTLESGVPSRFSGSGSRTDFTLTISSLQPEDFATYYCQQNNEDPLTFGQGTKLEIK

SEQ ID NO: 65 - protein, 111 aa, synthetic construct
  DOMAIN 1..111: note = hu127VL6
NIQLTQSPSSLSASVGQRVTITCRASESVDSYGNSFMHWYQQKPGKPPKVLIYLASTLESGVPSRFSGSGSRTDFTLTISSLQPEDFATYYCQQNNEDPLTFGQGTKLEIK

SEQ ID NO: 66 - protein, 119 aa, synthetic construct
  DOMAIN 1..119: note = hu128VH1
EVQLVQSGAEVKKPGASVKVSCKASGYTFTSYWMHWVRQAPGQGLEWMGRIDPNSGVTKYNEKFKSRVTMTVDKSTSTVYMELSSLRSEDTAVYYCARSSYLGRYFDVWGQGTTVTVSS

SEQ ID NO: 67 - protein, 119 aa, synthetic construct
  DOMAIN 1..119: note = hu128VH2
EVQLVQSGAEVKKPGASVKVSCKASGYTFTSYWMHWVRQAPGQGLEWMGRIDPNSGVTKYNEKFKSRVTMTVDKPSSTVYMELSSLRSEDTAVYYCARSSYLGRYFDVWGQGTTVTVSS

SEQ ID NO: 68 - protein, 119 aa, synthetic construct
  DOMAIN 1..119: note = hu128VH3
EVQLVQSGAEVKKPGASVKVSCKASGYTFTSYWMHWVRQAPGQGLEWMGRIDPNSGVTKYNEKFKSRVTLTVDKPSSPAYMELSSLRSEDTAVYYCARSSYLGRYFDVWGQGTTVTVSS

SEQ ID NO: 69 - protein, 119 aa, synthetic construct
  DOMAIN 1..119: note = hu128VH4
EVQLVQSGAEVKKPGASVKVSCKASGYTFTSYWMHWVRQRPGRGLEWMGRIDPNSGVTKYNEKFKSRVTLTVDKPSSPAYMELSSLRSEDTAVYYCARSSYLGRYFDVWGQGTTVTVSS

SEQ ID NO: 70 - protein, 106 aa, synthetic construct
  DOMAIN 1..106: note = hu128VL1
EIVLTQSPATLSLSPGERATLSCSATSSVSYMYWYQQKPGQAPRLLIYDTYNLASRIPARFSGSGSGTDYTLTISRLEPEDFAVYYCQQWSSYPPTFGQGTKLEIK

SEQ ID NO: 71 - protein, 106 aa, synthetic construct
  DOMAIN 1..106: note = hu128VL2
EIVLTQSPATLSLSPGERATLSCSATSSVSYMYWYQQKPGSSPRLLIYDTYNLASRIPARFSGSGSGTDYTLTISRLEPEDFAVYYCQQWSSYPPTFGQGTKLEIK

SEQ ID NO: 72 - protein, 106 aa, synthetic construct
  DOMAIN 1..106: note = hu128VL3
EIVLTQSPDFQSVTPKEKVTITCSATSSVSYMYWYQQKPDQSPKLLIYDTYNLASRVPSRFSGSGSGTDYTLTINSLEAEDAATYYCQQWSSYPPTFGQGTKLEIK

SEQ ID NO: 73 - protein, 7 aa, synthetic construct
  DOMAIN 1..7: note = hu128VL1-6-LCDR2
DTYNLGS

SEQ ID NO: 74 - protein, 106 aa, synthetic construct
  DOMAIN 1..106: note = hu128VL1-6
EIVLTQSPATLSLSPGERATLKCSATSSVSYMYWYQQKPGQAPRLLIYDTYNLGSRIPARFSGSGSGTDYTLTISRLEPEDFAVYYCQQWSSYPPTFGQGTKLEIK

SEQ ID NO: 75 - protein, 17 aa, synthetic construct
  DOMAIN 1..17: note = hu135VH3-HCDR2
YINSGGNYIYYADSVKG

SEQ ID NO: 76 - protein, 122 aa, synthetic construct
  DOMAIN 1..122: note = hu135VH1
DVKLVESGEGLVKPGGSLRLSCAASGFTFSTYGMSWVRQAPGKRLEWVAYINSGGNYIYYADTVKGRFTISRDNAKNSLYLQMNSLRAEDTAVYYCTRDRTTIVVHWYFDVWGQGTTVTVSS

SEQ ID NO: 77 - protein, 122 aa, synthetic construct
  DOMAIN 1..122: note = hu135VH2
DVKLVESGEGLVKPGGSLRLSCAASGFSISTYGMSWVRQAPGKRLEWVAYINSGGNYIYYADTVKGRFTISRDNAKNSLYLQMNSLRAEDTAVYYCTRDRTTIVVHWYFDVWGQGTTVTVSS

SEQ ID NO: 78 - protein, 122 aa, synthetic construct
  DOMAIN 1..122: note = hu135VH3
DVKLVESGEGLVKPGGSLRLSCAASGFSISTYGMSWVRQAPGKRLEWVAYINSGGNYIYYADSVKGRFTISRDNAKNSLYLQMNSLRAEDTAVYYCTRDRTTIVVHWYFDVWGQGTTVTVSS

SEQ ID NO: 79 - protein, 103 aa, synthetic construct
  DOMAIN 1..103: note = hu135VL1
DIQLTQSPSSLSASVGDRVTITCSASSSLNFMHWYQQKPGKSPKRWIYDTSKLASGVPSRFSGSGSGTDYTLTISSLQPEDFATYYCHQRSSTFGGGTKVEIK

SEQ ID NO: 80 - protein, 119 aa, synthetic construct
  DOMAIN 1..119: note = hu140VH3
EVQLVQSGAEVKKPGASVKVSCKASGYTFTSYWMHWVRQRPGRGLEWMGRIDPNSGVTKYNEKFKSRVTLTVDKPSSTAYMELSSLRSEDTAVYYCARSGGLRRYFDVWGQGTTVTVSS

SEQ ID NO: 81 - protein, 119 aa, synthetic construct
  DOMAIN 1..119: note = hu140VH4
QVQLVQSGAEVKKPGASVKVSCKASGYTFTSYWMHWVRQAPGQGLEWIGRIDPNSGVTKYNEKFKSRVTLTVDKPTSTAYIQLSSLRSEDTAVYYCARSGGLRRYFDVWGQGTTVTVSS

SEQ ID NO: 82 - protein, 119 aa, synthetic construct
  DOMAIN 1..119: note = hu140VH5
QVQLVQSGAEVKKPGASVKVSCKASGYTFTSYWMHWVRQAPGQGLEWMGRIDPNSGVTKYNEKFKSRVTLTVDKPSSPAYMELSSLRSEDTAVYYCARSGGLRRYFDVWGQGTTVTVSS

SEQ ID NO: 83 - protein, 106 aa, synthetic construct
  DOMAIN 1..106: note = hu140VL3
EIVLTQSPATLSLSPGERATLSCSASSSVSYMYWYQQKPGQAPRLLIYDTYNLASGVPARFSGSGSGTDYTLTISSLEPEDFAVYYCQQWSSYPPTFGQGTKLEIK

SEQ ID NO: 84 - protein, 106 aa, synthetic construct
  DOMAIN 1..106: note = hu140VL5
EIVLTQSPATLSLSPGERATLSCSASSSVSYMYWYQQKPGQAPRLLIYDTYNLASGVPARFSGSGSGTSYTLTISRLEPEDFAVYYCQQWSSYPPTFGAGTKLEIK

SEQ ID NO: 85 - protein, 106 aa, synthetic construct
  DOMAIN 1..106: note = hu140VL5-11
EIVLTQSPATLSLSPGERAQLSCSASSSVSYMYWYQQKPGQAPRLLIYDTYNLASGVPDRFSGSGSGTSYTLTISRLEPEDFAVYYCQQWSSYPPTFGAGTKLEIK

SEQ ID NO: 86 - protein, 330 aa, synthetic construct
  DOMAIN 1..330: note = IgG1 LALA
ASTKGPSVFPLAPSSKSTSGGTAALGCLVKDYFPEPVTVSWNSGALTSGVHTFPAVLQSSGLYSLSSVVTVPSSSLGTQTYICNVNHKPSNTKVDKKVEPKSCDKTHTCPPCPAPEAAGGPSVFLFPPKPKDTLMISRTPEVTCVVVDVSHEDPEVKFNWYVDGVEVHNAKTKPREEQYNSTYRVVSVLTVLHQDWLNGKEYKCKVSNKALPAPIEKTISKAKGQPREPQVYTLPPSRDELTKNQVSLTCLVKGFYPSDIAVEWESNGQPENNYKTTPPVLDSDGSFFLYSKLTVDKSRWQQGNVFSCSVMHEALHNHYTQKSLSLSPGK

SEQ ID NO: 87 - protein, 452 aa, synthetic construct
  CHAIN 1..452: note = Hu102H4L6-HC
DVKLVESGEGLVKPGGSLRLSCAASGFTFSSYAMSWVRQAPGKRLEWVAYISRGGDYIYYADSVKGRFTISRDNAKNSLYLQMNSLRAEDSAVYYCTRDQTTVVVHWYFDVWGQGTTVTVSSASTKGPSVFPLAPSSKSTSGGTAALGCLVKDYFPEPVTVSWNSGALTSGVHTFPAVLQSSGLYSLSSVVTVPSSSLGTQTYICNVNHKPSNTKVDKKVEPKSCDKTHTCPPCPAPEAAGGPSVFLFPPKPKDTLMISRTPEVTCVVVDVSHEDPEVKFNWYVDGVEVHNAKTKPREEQYNSTYRVVSVLTVLHQDWLNGKEYKCKVSNKALPAPIEKTISKAKGQPREPQVYTLPPSRDELTKNQVSLTCLVKGFYPSDIAVEWESNGQPENNYKTTPPVLDSDGSFFLYSKLTVDKSRWQQGNVFSCSVMHEALHNHYTQKSLSLSPGK

SEQ ID NO: 88 - protein, 211 aa, synthetic construct
  CHAIN 1..211: note = Hu102H4L6-LC
DIQLTQSPSSLSASVGDRVTITCSASSSINYMHWYQQKPGKSPKRWIYDTSKLASGVPSRFSGSGSGTDYTLTISSLQPEDFATYYCHQRNSYTFGGGTKVEIKRTVAAPSVFIFPPSDEQLKSGTASVVCLLNNFYPREAKVQWKVDNALQSGNSQESVTEQDSKDSTYSLSSTLTLSKADYEKHKVYACEVTHQGLSSPVTKSFNRGEC

SEQ ID NO: 89 - protein, 449 aa, synthetic construct
  CHAIN 1..449: note = Hu140H5L5-11-HC
QVQLVQSGAEVKKPGASVKVSCKASGYTFTSYWMHWVRQAPGQGLEWMGRIDPNSGVTKYNEKFKSRVTLTVDKPSSPAYMELSSLRSEDTAVYYCARSGGLRRYFDVWGQGTTVTVSSASTKGPSVFPLAPSSKSTSGGTAALGCLVKDYFPEPVTVSWNSGALTSGVHTFPAVLQSSGLYSLSSVVTVPSSSLGTQTYICNVNHKPSNTKVDKKVEPKSCDKTHTCPPCPAPEAAGGPSVFLFPPKPKDTLMISRTPEVTCVVVDVSHEDPEVKFNWYVDGVEVHNAKTKPREEQYNSTYRVVSVLTVLHQDWLNGKEYKCKVSNKALPAPIEKTISKAKGQPREPQVYTLPPSRDELTKNQVSLTCLVKGFYPSDIAVEWESNGQPENNYKTTPPVLDSDGSFFLYSKLTVDKSRWQQGNVFSCSVMHEALHNHYTQKSLSLSPGK

SEQ ID NO: 90 - protein, 213 aa, synthetic construct
  CHAIN 1..213: note = Hu140H5L5-11-LC
EIVLTQSPATLSLSPGERAQLSCSASSSVSYMYWYQQKPGQAPRLLIYDTYNLASGVPDRFSGSGSGTSYTLTISRLEPEDFAVYYCQQWSSYPPTFGAGTKLEIKRTVAAPSVFIFPPSDEQLKSGTASVVCLLNNFYPREAKVQWKVDNALQSGNSQESVTEQDSKDSTYSLSSTLTLSKADYEKHKVYACEVTHQGLSSPVTKSFNRGEC

SEQ ID NO: 91 - protein, 451 aa, synthetic construct
  CHAIN 1..451: note = REGN-5381-HC
QVQLVQSGAEVKKPGASVTVSCKASGYTFTDYYMHWVRQAPGQGLEWMGWIKPNSGGTNSAQRFQGRITMTWDTSISTAYMELSRLRSDDTAVYYCSRGGPVMNYYYYYGMDVWGQGTTVTVSSASTKGPSVFPLAPCSRSTSESTAALGCLVKDYFPEPVTVSWNSGALTSGVHTFPAVLQSSGLYSLSSVVTVPSSSLGTKTYTCNVDHKPSNTKVDKRVESKYGPPCPPCPAPEFLGGPSVFLFPPKPKDTLMISRTPEVTCVVVDVSQEDPEVQFNWYVDGVEVHNAKTKPREEQFNSTYRVVSVLTVLHQDWLNGKEYKCKVSNKGLPSSIEKTISKAKGQPREPQVYTLPPSQEEMTKNQVSLTCLVKGFYPSDIAVEWESNGQPENNYKTTPPVLDSDGSFFLYSRLTVDKSRWQEGNVFSCSVMHEALHNHYTQKSLSLSLGK

SEQ ID NO: 92 - protein, 213 aa, synthetic construct
  CHAIN 1..213: note = REGN-5381-LC
NIQMTQSPSSLSASVGDRVTITCRASQSIDSYLNWYQQKPGKAPKLLIYVASSLQSGVPSRFSGSGSGKDFTLTISSLQPEDFATYYCQQSYSIPTFGQGTRLEIKRTVAAPSVFIFPPSDEQLKSGTASVVCLLNNFYPREAKVQWKVDNALQSGNSQESVTEQDSKDSTYSLSSTLTLSKADYEKHKVYACEVTHQGLSSPVTKSFNRGEC

SEQ ID NO: 93 - protein, 454 aa, synthetic construct
  CHAIN 1..454: note = REGN-5381-m-HC
QVQLVQSGAEVKKPGASVTVSCKASGYTFTDYYMHWVRQAPGQGLEWMGWIKPNSGGTNSAQRFQGRITMTWDTSISTAYMELSRLRSDDTAVYYCSRGGPVMNYYYYYGMDVWGQGTTVTVSSAKTTAPSVYPLAPVCGDTTGSSVTLGCLVKGYFPEPVTLTWNSGSLSSGVHTFPAVLQSDLYTLSSSVTVTSSTWPSQSITCNVAHPASSTKVDKKIEPRGPTIKPCPPCKCPAPNLLGGPSVFIFPPKIKDVLMISLSPIVTCVVVDVSEDDPDVQISWFVNNVEVHTAQTQTHREDYNSTLRVVSALPIQHQDWMSGKEFKCKVNNKDLPAPIERTISKPKGSVRAPQVYVLPPPEEEMTKKQVTLTCMVTDFMPEDIYVEWTNNGKTELNYKNTEPVLDSDGSYFMYSKLRVEKKNWVERNSYSCSVVHEGLHNHHTTKSFSRTPGK

SEQ ID NO: 94 - protein, 213 aa, synthetic construct
  CHAIN 1..213: note = REGN-5381-m-LC
NIQMTQSPSSLSASVGDRVTITCRASQSIDSYLNWYQQKPGKAPKLLIYVASSLQSGVPSRFSGSGSGKDFTLTISSLQPEDFATYYCQQSYSIPTFGQGTRLEIKRADAAPTVSIFPPSSEQLTSGGASVVCFLNNFYPKDINVKWKIDGSERQNGVLNSWTDQDSKDSTYSMSSTLTLTKDEYERHNSYTCEATHKTSTSPIVKSFNRNEC

SEQ ID NO: 95 - protein, 455 aa, synthetic construct
  CHAIN 1..455: note = XX16 V-HC
QVQLLESGGGLVQPGGSLRLSCAASGFTFSSYWMNWVRQAPGKGLEWVSVIESKGNYIFYADSVKGRFTISRDNSKNTLYLQMNSLRAEDTAVYYCARDRYSMIYSYGAGAFDYWGQGTLVTVSSASTKGPSVFPLAPSSKSTSGGTAALGCLVKDYFPEPVTVSWNSGALTSGVHTFPAVLQSSGLYSLSSVVTVPSSSLGTQTYICNVNHKPSNTKVDKKVEPKSCDKTHTCPPCPAPEAAGGPSVFLFPPKPKDTLMISRTPEVTCVVVDVSHEDPEVKFNWYVDGVEVHNAKTKPREEQYNSTYRVVSVLTVLHQDWLNGKEYKCKVSNKALPAPIEKTISKAKGQPREPQVYTLPPSRDELTKNQVSLTCLVKGFYPSDIAVEWESNGQPENNYKTTPPVLDSDGSFFLYSKLTVDKSRWQQGNVFSCSVMHEALHNHYTQKSLSLSPGK

SEQ ID NO: 96 - protein, 214 aa, synthetic construct
  CHAIN 1..214: note = XX16 V-LC
DIQMTQSPSSLSASVGDRVTITCRASQGISSYLAWYQQKPGKAPKLLIYTASTLQSGVPSRFSGSGSGTDFTLTISSLQPEDFATYYCQQTWRKPRTFGQGTKVEIKRTVAAPSVFIFPPSDEQLKSGTASVVCLLNNFYPREAKVQWKVDNALQSGNSQESVTEQDSKDSTYSLSSTLTLSKADYEKHKVYACEVTHQGLSSPVTKSFNRGEC

SEQ ID NO: 97 - protein, 444 aa, synthetic construct
  CHAIN 1..444: note = RC25 V-HC
QVQLVQSGAEVKKPGASVKVSCKASGYTFTNSWIGWFRQAPGQGLEWIGDIYPGGGYTNYNEIFKGKATMTADTSTNTAYMELSSLRSEDTAVYYCSRGIPGYAMDYWGQGTLVTVSSASTKGPSVFPLAPCSRSTSESTAALGCLVKDYFPEPVTVSWNSGALTSGVHTFPAVLQSSGLYSLSSVVTVPSSSLGTKTYTCNVDHKPSNTKVDKRVESKYGPPCPPCPAPEFLGGPSVFLFPPKPKDTLMISRTPEVTCVVVDVSQEDPEVQFNWYVDGVEVHNAKTKPREEQFNSTYRVVSVLTVLHQDWLNGKEYKCKVSNKGLPSSIEKTISKAKGQPREPQVYTLPPSQEEMTKNQVSLTCLVKGFYPSDIAVEWESNGQPENNYKTTPPVLDSDGSFFLYSRLTVDKSRWQEGNVFSCSVMHEALHNHYTQKSLSLSLG

SEQ ID NO: 98 - protein, 220 aa, synthetic construct
  CHAIN 1..220: note = RC25 V-LC
DIQMTQSPSSLSASVGDRVTMSCKSSQSLLNSGDQKNYLTWYQQKPGKAPKLLIYWASTGESGVPSRFSGSGSGTDFTFTISSLQPEDIATYYCQNDYSYPWTFGQGTKVEIKRTVAAPSVFIFPPSDEQLKSGTASVVCLLNNFYPREAKVQWKVDNALQSGNSQESVTEQDSKDSTYSLSSTLTLSKADYEKHKVYACEVTHQGLSSPVTKSFNRGEC

SEQ ID NO: 99 - protein, 449 aa, synthetic construct
  CHAIN 1..449: note = Hu128H3L1-6-HC
EVQLVQSGAEVKKPGASVKVSCKASGYTFTSYWMHWVRQAPGQGLEWMGRIDPNSGVTKYNEKFKSRVTLTVDKPSSPAYMELSSLRSEDTAVYYCARSSYLGRYFDVWGQGTTVTVSSASTKGPSVFPLAPSSKSTSGGTAALGCLVKDYFPEPVTVSWNSGALTSGVHTFPAVLQSSGLYSLSSVVTVPSSSLGTQTYICNVNHKPSNTKVDKKVEPKSCDKTHTCPPCPAPEAAGGPSVFLFPPKPKDTLMISRTPEVTCVVVDVSHEDPEVKFNWYVDGVEVHNAKTKPREEQYNSTYRVVSVLTVLHQDWLNGKEYKCKVSNKALPAPIEKTISKAKGQPREPQVYTLPPSRDELTKNQVSLTCLVKGFYPSDIAVEWESNGQPENNYKTTPPVLDSDGSFFLYSKLTVDKSRWQQGNVFSCSVMHEALHNHYTQKSLSLSPGK

SEQ ID NO: 100 - protein, 213 aa, synthetic construct
  CHAIN 1..213: note = Hu128H3L1-6-LC
EIVLTQSPATLSLSPGERATLKCSATSSVSYMYWYQQKPGQAPRLLIYDTYNLGSRIPARFSGSGSGTDYTLTISRLEPEDFAVYYCQQWSSYPPTFGQGTKLEIKRTVAAPSVFIFPPSDEQLKSGTASVVCLLNNFYPREAKVQWKVDNALQSGNSQESVTEQDSKDSTYSLSSTLTLSKADYEKHKVYACEVTHQGLSSPVTKSFNRGEC

SEQ ID NO: 101 - protein, 452 aa, synthetic construct
  CHAIN 1..452: note = Hu135H3L1-HC
DVKLVESGEGLVKPGGSLRLSCAASGFSISTYGMSWVRQAPGKRLEWVAYINSGGNYIYYADSVKGRFTISRDNAKNSLYLQMNSLRAEDTAVYYCTRDRTTIVVHWYFDVWGQGTTVTVSSASTKGPSVFPLAPSSKSTSGGTAALGCLVKDYFPEPVTVSWNSGALTSGVHTFPAVLQSSGLYSLSSVVTVPSSSLGTQTYICNVNHKPSNTKVDKKVEPKSCDKTHTCPPCPAPEAAGGPSVFLFPPKPKDTLMISRTPEVTCVVVDVSHEDPEVKFNWYVDGVEVHNAKTKPREEQYNSTYRVVSVLTVLHQDWLNGKEYKCKVSNKALPAPIEKTISKAKGQPREPQVYTLPPSRDELTKNQVSLTCLVKGFYPSDIAVEWESNGQPENNYKTTPPVLDSDGSFFLYSKLTVDKSRWQQGNVFSCSVMHEALHNHYTQKSLSLSPGK

SEQ ID NO: 102 - protein, 452 aa, synthetic construct
  CHAIN 1..452: note = CHI-102-heavy chain
DVKLVESGEGLVKPGGSLKLSCAASGFTFSTYAMSWVRQTPEKRLEWVAYISRGGDYIYYADTVKGRFTISRDNARNTLYLQMSSLKSEDTAMYYCTRDQTTVVVHWYFDVWGTGTTVTVSSASTKGPSVFPLAPSSKSTSGGTAALGCLVKDYFPEPVTVSWNSGALTSGVHTFPAVLQSSGLYSLSSVVTVPSSSLGTQTYICNVNHKPSNTKVDKKVEPKSCDKTHTCPPCPAPELLGGPSVFLFPPKPKDTLMISRTPEVTCVVVDVSHEDPEVKFNWYVDGVEVHNAKTKPREEQYNSTYRVVSVLTVLHQDWLNGKEYKCKVSNKALPAPIEKTISKAKGQPREPQVYTLPPSRDELTKNQVSLTCLVKGFYPSDIAVEWESNGQPENNYKTTPPVLDSDGSFFLYSKLTVDKSRWQQGNVFSCSVMHEALHNHYTQKSLSLSPGK

SEQ ID NO: 103 - protein, 211 aa, synthetic construct
  CHAIN 1..211: note = CHI-102-light chain
QIVLTQSPAIMSASPGEKVTMTCSASSSINYMHWYQQKPGTSPKRWIYDTSKLASGVPARFSGSGSGTSYSLTISSMEAGDAATYYCHQRNSYTFGGGTKLEIKRTVAAPSVFIFPPSDEQLKSGTASVVCLLNNFYPREAKVQWKVDNALQSGNSQESVTEQDSKDSTYSLSSTLTLSKADYEKHKVYACEVTHQGLSSPVTKSFNRGEC

SEQ ID NO: 104 - protein, 452 aa, synthetic construct
  CHAIN 1..452: note = CHI-127-heavy chain
QAYLQQSGPELVKPGASVKISCKASGYSFTGYFMNWVMQSHGKSLEWIGRINPYNGDTFYNQKFKGKATLTVDKSSSTVHMELRSLASEDSAVYYCARRGYGNRGYWYFDVWGAGTTVTVSSASTKGPSVFPLAPSSKSTSGGTAALGCLVKDYFPEPVTVSWNSGALTSGVHTFPAVLQSSGLYSLSSVVTVPSSSLGTQTYICNVNHKPSNTKVDKKVEPKSCDKTHTCPPCPAPELLGGPSVFLFPPKPKDTLMISRTPEVTCVVVDVSHEDPEVKFNWYVDGVEVHNAKTKPREEQYNSTYRVVSVLTVLHQDWLNGKEYKCKVSNKALPAPIEKTISKAKGQPREPQVYTLPPSRDELTKNQVSLTCLVKGFYPSDIAVEWESNGQPENNYKTTPPVLDSDGSFFLYSKLTVDKSRWQQGNVFSCSVMHEALHNHYTQKSLSLSPGK

SEQ ID NO: 105 - protein, 218 aa, synthetic construct
  CHAIN 1..218: note = CHI-127-light chain
NIVLTQSPASLAVSLGQRATISCRASESVDSYGNSFMHWYQQKPGQPPKVLIYLASTLESGVPARFSGSGSRTDFTLTIDPVEADDAATYYCQQNNEDPLTFGAGTKLELKRTVAAPSVFIFPPSDEQLKSGTASVVCLLNNFYPREAKVQWKVDNALQSGNSQESVTEQDSKDSTYSLSSTLTLSKADYEKHKVYACEVTHQGLSSPVTKSFNRGEC

SEQ ID NO: 106 - protein, 449 aa, synthetic construct
  CHAIN 1..449: note = CHI-128-heavy chain
QVQLQQSGAELAKPGASVKLSCKASGYTFTSYWMHWVKQRPGRGLEWIGRIDPNSGVTKYNEKFKSKATLTVDKPSSPAYMQLSSLTSEDSAVYYCARSSYLGRYFDVWGTGTTVTVSSASTKGPSVFPLAPSSKSTSGGTAALGCLVKDYFPEPVTVSWNSGALTSGVHTFPAVLQSSGLYSLSSVVTVPSSSLGTQTYICNVNHKPSNTKVDKKVEPKSCDKTHTCPPCPAPELLGGPSVFLFPPKPKDTLMISRTPEVTCVVVDVSHEDPEVKFNWYVDGVEVHNAKTKPREEQYNSTYRVVSVLTVLHQDWLNGKEYKCKVSNKALPAPIEKTISKAKGQPREPQVYTLPPSRDELTKNQVSLTCLVKGFYPSDIAVEWESNGQPENNYKTTPPVLDSDGSFFLYSKLTVDKSRWQQGNVFSCSVMHEALHNHYTQKSLSLSPGK

SEQ ID NO: 107 - protein, 213 aa, synthetic construct
  CHAIN 1..213: note = CHI-128-light chain
QIVLTQSPAIMSASPGEKVTMTCSATSSVSYMYWYQQKPGSSPRLLIYDTYNLASRVPIRFSGSGSGTSYSLTISRMEAEDAATYYCQQWSSYPPTFGSGTKLEIKRTVAAPSVFIFPPSDEQLKSGTASVVCLLNNFYPREAKVQWKVDNALQSGNSQESVTEQDSKDSTYSLSSTLTLSKADYEKHKVYACEVTHQGLSSPVTKSFNRGEC

SEQ ID NO: 108 - protein, 452 aa, synthetic construct
  CHAIN 1..452: note = CHI-135-heavy chain
DVKLVESGEGLVKPGGSLKLSCVASGFSISTYGMSWVRQTPEKRLEWVAYINSGGNYIYYADTVKGRFTISRDNARNTLYLQMSSLKSEDTAMYYCTRDRTTIVVHWYFDVWGTGTTVTVSSASTKGPSVFPLAPSSKSTSGGTAALGCLVKDYFPEPVTVSWNSGALTSGVHTFPAVLQSSGLYSLSSVVTVPSSSLGTQTYICNVNHKPSNTKVDKKVEPKSCDKTHTCPPCPAPELLGGPSVFLFPPKPKDTLMISRTPEVTCVVVDVSHEDPEVKFNWYVDGVEVHNAKTKPREEQYNSTYRVVSVLTVLHQDWLNGKEYKCKVSNKALPAPIEKTISKAKGQPREPQVYTLPPSRDELTKNQVSLTCLVKGFYPSDIAVEWESNGQPENNYKTTPPVLDSDGSFFLYSKLTVDKSRWQQGNVFSCSVMHEALHNHYTQKSLSLSPGK

SEQ ID NO: 109 - protein, 210 aa, synthetic construct
  CHAIN 1..210: note = CHI-135-light chain
QIVLTQSPAIMSASPGEKVTMTCSASSSLNFMHWYQQKPGTSPKRWIYDTSKLASGVPARFSGSGSGTSYSLTISSMEAEDAATYYCHQRSSTFGGGTKLELKRTVAAPSVFIFPPSDEQLKSGTASVVCLLNNFYPREAKVQWKVDNALQSGNSQESVTEQDSKDSTYSLSSTLTLSKADYEKHKVYACEVTHQGLSSPVTKSFNRGEC

SEQ ID NO: 110 - protein, 449 aa, synthetic construct
  CHAIN 1..449: note = CHI-140 heavy chain
QVQLQQSGAELVKPGASVKLSCKASGYTFTSYWMHWVKQRPGRGLEWIGRIDPNSGVTKYNEKFKSKVTLTVDKPSSPAYIQLSSLTSEDSAVYYCARSGGLRRYFDVWGTGTTVTVSSASTKGPSVFPLAPSSKSTSGGTAALGCLVKDYFPEPVTVSWNSGALTSGVHTFPAVLQSSGLYSLSSVVTVPSSSLGTQTYICNVNHKPSNTKVDKKVEPKSCDKTHTCPPCPAPELLGGPSVFLFPPKPKDTLMISRTPEVTCVVVDVSHEDPEVKFNWYVDGVEVHNAKTKPREEQYNSTYRVVSVLTVLHQDWLNGKEYKCKVSNKALPAPIEKTISKAKGQPREPQVYTLPPSRDELTKNQVSLTCLVKGFYPSDIAVEWESNGQPENNYKTTPPVLDSDGSFFLYSKLTVDKSRWQQGNVFSCSVMHEALHNHYTQKSLSLSPGK

SEQ ID NO: 111 - protein, 213 aa, synthetic construct
  CHAIN 1..213: note = CHI-140-light chain
QIVLTQSPAIMSASPGEKVTMTCSASSSVSYMYWYQQKPGSSPRLLIFDTYNLASGVPVRFSGSGSGTSYSLTINRMEAEDAATYYCQQWSSYPPTFGAGTKLELKRTVAAPSVFIFPPSDEQLKSGTASVVCLLNNFYPREAKVQWKVDNALQSGNSQESVTEQDSKDSTYSLSSTLTLSKADYEKHKVYACEVTHQGLSSPVTKSFNRGEC

SEQ ID NO: 112 - protein, 452 aa, synthetic construct
  CHAIN 1..452: note = Hu102H2L6-heavy chain
EVQLVESGEGLVKPGGSLRLSCAASGFTFSTYAMSWVRQAPGKRLEWVAYISRGGDYIYYADTVKGRFTISRDNAKNSLYLQMNSLRAEDTAVYYCTRDQTTVVVHWYFDVWGQGTTVTVSSASTKGPSVFPLAPSSKSTSGGTAALGCLVKDYFPEPVTVSWNSGALTSGVHTFPAVLQSSGLYSLSSVVTVPSSSLGTQTYICNVNHKPSNTKVDKKVEPKSCDKTHTCPPCPAPEAAGGPSVFLFPPKPKDTLMISRTPEVTCVVVDVSHEDPEVKFNWYVDGVEVHNAKTKPREEQYNSTYRVVSVLTVLHQDWLNGKEYKCKVSNKALPAPIEKTISKAKGQPREPQVYTLPPSRDELTKNQVSLTCLVKGFYPSDIAVEWESNGQPENNYKTTPPVLDSDGSFFLYSKLTVDKSRWQQGNVFSCSVMHEALHNHYTQKSLSLSPGK

SEQ ID NO: 113 - protein, 452 aa, synthetic construct
  CHAIN 1..452: note = Hu102H3L6 heavy chain
DVKLVESGEGLVKPGGSLRLSCAASGFTFSTYAMSWVRQAPGKRLEWVAYISRGGDYIYYADTVKGRFTISRDNAKNSLYLQMNSLRAEDTAVYYCTRDQTTVVVHWYFDVWGQGTTVTVSSASTKGPSVFPLAPSSKSTSGGTAALGCLVKDYFPEPVTVSWNSGALTSGVHTFPAVLQSSGLYSLSSVVTVPSSSLGTQTYICNVNHKPSNTKVDKKVEPKSCDKTHTCPPCPAPEAAGGPSVFLFPPKPKDTLMISRTPEVTCVVVDVSHEDPEVKFNWYVDGVEVHNAKTKPREEQYNSTYRVVSVLTVLHQDWLNGKEYKCKVSNKALPAPIEKTISKAKGQPREPQVYTLPPSRDELTKNQVSLTCLVKGFYPSDIAVEWESNGQPENNYKTTPPVLDSDGSFFLYSKLTVDKSRWQQGNVFSCSVMHEALHNHYTQKSLSLSPGK

SEQ ID NO: 114 - protein, 452 aa, synthetic construct
  CHAIN 1..452: note = Hu102H5L6 heavy chain
DVKLVESGEGLVKPGGSLRLSCAASGFTFSTYGMSWVRQAPGKRLEWVAYISRGGDYIYYADTVKGRFTISRDNAKNSLYLQMNSLRAEDTAVYYCTRDQTTVVVHWYFDVWGQGTTVTVSSASTKGPSVFPLAPSSKSTSGGTAALGCLVKDYFPEPVTVSWNSGALTSGVHTFPAVLQSSGLYSLSSVVTVPSSSLGTQTYICNVNHKPSNTKVDKKVEPKSCDKTHTCPPCPAPEAAGGPSVFLFPPKPKDTLMISRTPEVTCVVVDVSHEDPEVKFNWYVDGVEVHNAKTKPREEQYNSTYRVVSVLTVLHQDWLNGKEYKCKVSNKALPAPIEKTISKAKGQPREPQVYTLPPSRDELTKNQVSLTCLVKGFYPSDIAVEWESNGQPENNYKTTPPVLDSDGSFFLYSKLTVDKSRWQQGNVFSCSVMHEALHNHYTQKSLSLSPGK

SEQ ID NO: 115 - protein, 452 aa, synthetic construct
  CHAIN 1..452: note = Hu127H4L1 heavy chain
EAYLVQSGAEVKKPGASVKVSCKASGYSFTGYFMNWVRQAPGKGLEWMGRINPYSGDTFYNQKFKGRVTLTVDKSTSTVYMELSSLRSEDTAVYYCARRGYGNRGYWYFDVWGQGTTVTVSSASTKGPSVFPLAPSSKSTSGGTAALGCLVKDYFPEPVTVSWNSGALTSGVHTFPAVLQSSGLYSLSSVVTVPSSSLGTQTYICNVNHKPSNTKVDKKVEPKSCDKTHTCPPCPAPEAAGGPSVFLFPPKPKDTLMISRTPEVTCVVVDVSHEDPEVKFNWYVDGVEVHNAKTKPREEQYNSTYRVVSVLTVLHQDWLNGKEYKCKVSNKALPAPIEKTISKAKGQPREPQVYTLPPSRDELTKNQVSLTCLVKGFYPSDIAVEWESNGQPENNYKTTPPVLDSDGSFFLYSKLTVDKSRWQQGNVFSCSVMHEALHNHYTQKSLSLSPGK

SEQ ID NO: 116 - protein, 452 aa, synthetic construct
  CHAIN 1..452: note = Hu127H7L1 heavy chain
QVQLVQSGAEVKKPGASVKVSCKASGYTFTGYFMNWVRQAPGQGLEWMGRINPYSGDTFYNQKFKGRVTMTVDKSTSTVYMELSSLRSEDTAVYYCARRGYGNRGYWYFDVWGQGTTVTVSSASTKGPSVFPLAPSSKSTSGGTAALGCLVKDYFPEPVTVSWNSGALTSGVHTFPAVLQSSGLYSLSSVVTVPSSSLGTQTYICNVNHKPSNTKVDKKVEPKSCDKTHTCPPCPAPEAAGGPSVFLFPPKPKDTLMISRTPEVTCVVVDVSHEDPEVKFNWYVDGVEVHNAKTKPREEQYNSTYRVVSVLTVLHQDWLNGKEYKCKVSNKALPAPIEKTISKAKGQPREPQVYTLPPSRDELTKNQVSLTCLVKGFYPSDIAVEWESNGQPENNYKTTPPVLDSDGSFFLYSKLTVDKSRWQQGNVFSCSVMHEALHNHYTQKSLSLSPGK

SEQ ID NO: 117 - protein, 452 aa, synthetic construct
  CHAIN 1..452: note = Hu127H8L1 heavy chain
EVQLVQSGAEVKKPGASVKVSCKASGYTFTGYFMNWVRQAPGQGLEWMGRINPYSGDTFYNQKFKGRVTMTVDKSTSTVYMELSSLRSEDTAVYYCARRGYGNRGYWYFDVWGQGTTVTVSSASTKGPSVFPLAPSSKSTSGGTAALGCLVKDYFPEPVTVSWNSGALTSGVHTFPAVLQSSGLYSLSSVVTVPSSSLGTQTYICNVNHKPSNTKVDKKVEPKSCDKTHTCPPCPAPEAAGGPSVFLFPPKPKDTLMISRTPEVTCVVVDVSHEDPEVKFNWYVDGVEVHNAKTKPREEQYNSTYRVVSVLTVLHQDWLNGKEYKCKVSNKALPAPIEKTISKAKGQPREPQVYTLPPSRDELTKNQVSLTCLVKGFYPSDIAVEWESNGQPENNYKTTPPVLDSDGSFFLYSKLTVDKSRWQQGNVFSCSVMHEALHNHYTQKSLSLSPGK

SEQ ID NO: 118 - protein, 218 aa, synthetic construct
  CHAIN 1..218: note = Hu127H4L1_light chain
DIVMTQSPDSLAVSLGERATINCRASESVDSYGNSFMHWYQQKPGQPPKVLIYLASTLESGVPDRFSGSGSRTDFTLTISSLQAEDVAVYYCQQNNEDPLTFGQGTKLEIKRTVAAPSVFIFPPSDEQLKSGTASVVCLLNNFYPREAKVQWKVDNALQSGNSQESVTEQDSKDSTYSLSSTLTLSKADYEKHKVYACEVTHQGLSSPVTKSFNRGEC

SEQ ID NO: 119 - protein, 218 aa, synthetic construct
  CHAIN 1..218: note = Hu127H4L3-light chain
NIVLTQSPDSLAVSLGERATINCRASESVDSYGNSFMHWYQQKPGQPPKVLIYLASTLESGVPDRFSGSGSRTDFTLTISSLQAEDVAVYYCQQNNEDPLTFGQGTKLEIKRTVAAPSVFIFPPSDEQLKSGTASVVCLLNNFYPREAKVQWKVDNALQSGNSQESVTEQDSKDSTYSLSSTLTLSKADYEKHKVYACEVTHQGLSSPVTKSFNRGEC

SEQ ID NO: 120 - protein, 218 aa, synthetic construct
  CHAIN 1..218: note = Hu127H4L5-light chain
NIQLTQSPSSLSASVGDRVTITCRASESVDSYGNSFMHWYQQKPGKAPKVLIYLASTLESGVPSRFSGSGSRTDFTLTISSLQPEDFATYYCQQNNEDPLTFGQGTKLEIKRTVAAPSVFIFPPSDEQLKSGTASVVCLLNNFYPREAKVQWKVDNALQSGNSQESVTEQDSKDSTYSLSSTLTLSKADYEKHKVYACEVTHQGLSSPVTKSFNRGEC

SEQ ID NO: 121 - protein, 218 aa, synthetic construct
  CHAIN 1..218: note = Hu127H4L6-light chain
NIQLTQSPSSLSASVGQRVTITCRASESVDSYGNSFMHWYQQKPGKPPKVLIYLASTLESGVPSRFSGSGSRTDFTLTISSLQPEDFATYYCQQNNEDPLTFGQGTKLEIKRTVAAPSVFIFPPSDEQLKSGTASVVCLLNNFYPREAKVQWKVDNALQSGNSQESVTEQDSKDSTYSLSSTLTLSKADYEKHKVYACEVTHQGLSSPVTKSFNRGEC

SEQ ID NO: 122 - protein, 449 aa, synthetic construct
  CHAIN 1..449: note = Hu128H2L1 heavy chain
EVQLVQSGAEVKKPGASVKVSCKASGYTFTSYWMHWVRQAPGQGLEWMGRIDPNSGVTKYNEKFKSRVTMTVDKPSSTVYMELSSLRSEDTAVYYCARSSYLGRYFDVWGQGTTVTVSSASTKGPSVFPLAPSSKSTSGGTAALGCLVKDYFPEPVTVSWNSGALTSGVHTFPAVLQSSGLYSLSSVVTVPSSSLGTQTYICNVNHKPSNTKVDKKVEPKSCDKTHTCPPCPAPEAAGGPSVFLFPPKPKDTLMISRTPEVTCVVVDVSHEDPEVKFNWYVDGVEVHNAKTKPREEQYNSTYRVVSVLTVLHQDWLNGKEYKCKVSNKALPAPIEKTISKAKGQPREPQVYTLPPSRDELTKNQVSLTCLVKGFYPSDIAVEWESNGQPENNYKTTPPVLDSDGSFFLYSKLTVDKSRWQQGNVFSCSVMHEALHNHYTQKSLSLSPGK

SEQ ID NO: 123 - protein, 213 aa, synthetic construct
  CHAIN 1..213: note = Hu128H2L1-light chain
EIVLTQSPATLSLSPGERATLSCSATSSVSYMYWYQQKPGQAPRLLIYDTYNLASRIPARFSGSGSGTDYTLTISRLEPEDFAVYYCQQWSSYPPTFGQGTKLEIKRTVAAPSVFIFPPSDEQLKSGTASVVCLLNNFYPREAKVQWKVDNALQSGNSQESVTEQDSKDSTYSLSSTLTLSKADYEKHKVYACEVTHQGLSSPVTKSFNRGEC

SEQ ID NO: 124 - protein, 213 aa, synthetic construct
  CHAIN 1..213: note = Hu128H2L2-light chain
EIVLTQSPATLSLSPGERATLSCSATSSVSYMYWYQQKPGSSPRLLIYDTYNLASRIPARFSGSGSGTDYTLTISRLEPEDFAVYYCQQWSSYPPTFGQGTKLEIKRTVAAPSVFIFPPSDEQLKSGTASVVCLLNNFYPREAKVQWKVDNALQSGNSQESVTEQDSKDSTYSLSSTLTLSKADYEKHKVYACEVTHQGLSSPVTKSFNRGEC

SEQ ID NO: 125 - protein, 452 aa, synthetic construct
  CHAIN 1..452: note = Hu135H1L1 heavy chain
DVKLVESGEGLVKPGGSLRLSCAASGFTFSTYGMSWVRQAPGKRLEWVAYINSGGNYIYYADTVKGRFTISRDNAKNSLYLQMNSLRAEDTAVYYCTRDRTTIVVHWYFDVWGQGTTVTVSSASTKGPSVFPLAPSSKSTSGGTAALGCLVKDYFPEPVTVSWNSGALTSGVHTFPAVLQSSGLYSLSSVVTVPSSSLGTQTYICNVNHKPSNTKVDKKVEPKSCDKTHTCPPCPAPEAAGGPSVFLFPPKPKDTLMISRTPEVTCVVVDVSHEDPEVKFNWYVDGVEVHNAKTKPREEQYNSTYRVVSVLTVLHQDWLNGKEYKCKVSNKALPAPIEKTISKAKGQPREPQVYTLPPSRDELTKNQVSLTCLVKGFYPSDIAVEWESNGQPENNYKTTPPVLDSDGSFFLYSKLTVDKSRWQQGNVFSCSVMHEALHNHYTQKSLSLSPGK

SEQ ID NO: 126 - protein, 452 aa, synthetic construct
  CHAIN 1..452: note = Hu135H2L1-heavy chain
DVKLVESGEGLVKPGGSLRLSCAASGFSISTYGMSWVRQAPGKRLEWVAYINSGGNYIYYADTVKGRFTISRDNAKNSLYLQMNSLRAEDTAVYYCTRDRTTIVVHWYFDVWGQGTTVTVSSASTKGPSVFPLAPSSKSTSGGTAALGCLVKDYFPEPVTVSWNSGALTSGVHTFPAVLQSSGLYSLSSVVTVPSSSLGTQTYICNVNHKPSNTKVDKKVEPKSCDKTHTCPPCPAPEAAGGPSVFLFPPKPKDTLMISRTPEVTCVVVDVSHEDPEVKFNWYVDGVEVHNAKTKPREEQYNSTYRVVSVLTVLHQDWLNGKEYKCKVSNKALPAPIEKTISKAKGQPREPQVYTLPPSRDELTKNQVSLTCLVKGFYPSDIAVEWESNGQPENNYKTTPPVLDSDGSFFLYSKLTVDKSRWQQGNVFSCSVMHEALHNHYTQKSLSLSPGK

SEQ ID NO: 127 - protein, 449 aa, synthetic construct
  CHAIN 1..449: note = Hu140H4L5-heavy chain
QVQLVQSGAEVKKPGASVKVSCKASGYTFTSYWMHWVRQAPGQGLEWIGRIDPNSGVTKYNEKFKSRVTLTVDKPTSTAYIQLSSLRSEDTAVYYCARSGGLRRYFDVWGQGTTVTVSSASTKGPSVFPLAPSSKSTSGGTAALGCLVKDYFPEPVTVSWNSGALTSGVHTFPAVLQSSGLYSLSSVVTVPSSSLGTQTYICNVNHKPSNTKVDKKVEPKSCDKTHTCPPCPAPEAAGGPSVFLFPPKPKDTLMISRTPEVTCVVVDVSHEDPEVKFNWYVDGVEVHNAKTKPREEQYNSTYRVVSVLTVLHQDWLNGKEYKCKVSNKALPAPIEKTISKAKGQPREPQVYTLPPSRDELTKNQVSLTCLVKGFYPSDIAVEWESNGQPENNYKTTPPVLDSDGSFFLYSKLTVDKSRWQQGNVFSCSVMHEALHNHYTQKSLSLSPGK

SEQ ID NO: 128 - protein, 213 aa, synthetic construct
  CHAIN 1..213: note = Hu140H4L5-light chain
EIVLTQSPATLSLSPGERATLSCSASSSVSYMYWYQQKPGQAPRLLIYDTYNLASGVPARFSGSGSGTSYTLTISRLEPEDFAVYYCQQWSSYPPTFGAGTKLEIKRTVAAPSVFIFPPSDEQLKSGTASVVCLLNNFYPREAKVQWKVDNALQSGNSQESVTEQDSKDSTYSLSSTLTLSKADYEKHKVYACEVTHQGLSSPVTKSFNRGEC